European Patent Specification EP 3 157 565 B1, published April 24, 2024. Title: TREATMENT OF POLYBACTERIAL INFECTIONS. Applicant: MEDIMMUNE, LLC. Application To Be Assigned. The sequence listing filed with the application follows.

SEQUENCE LISTING (101 sequences)

SEQ ID NO: 1 - protein, 11 aa, Artificial Sequence
  Description of Artificial Sequence: Synthetic peptide
RASQSISSWLA

SEQ ID NO: 2 - protein, 7 aa, Artificial Sequence
  Description of Artificial Sequence: Synthetic peptide
KASSLES

SEQ ID NO: 3 - protein, 8 aa, Artificial Sequence
  Description of Artificial Sequence: Synthetic peptide
QQYNSYWT

SEQ ID NO: 4 - protein, 11 aa, Artificial Sequence
  Description of Artificial Sequence: Synthetic peptide
RASQGIRNDLG

SEQ ID NO: 5 - protein, 7 aa, Artificial Sequence
  Description of Artificial Sequence: Synthetic peptide
DASSLQS

SEQ ID NO: 6 - protein, 9 aa, Artificial Sequence
  Description of Artificial Sequence: Synthetic peptide
LQDYNYPWT

SEQ ID NO: 7 - protein, 5 aa, Artificial Sequence
  Description of Artificial Sequence: Synthetic peptide
SYDMH

SEQ ID NO: 8 - protein, 16 aa, Artificial Sequence
  Description of Artificial Sequence: Synthetic peptide
GIGTAGDTYYPGSVKG

SEQ ID NO: 9 - protein, 14 aa, Artificial Sequence
  Description of Artificial Sequence: Synthetic peptide
DNYSSTGGYYGMDV

SEQ ID NO: 10 - protein, 5 aa, Artificial Sequence
  Description of Artificial Sequence: Synthetic peptide
RYDMH

SEQ ID NO: 11 - protein, 16 aa, Artificial Sequence
  Description of Artificial Sequence: Synthetic peptide
VIGTDGDTYYPGSVKG

SEQ ID NO: 12 - protein, 14 aa, Artificial Sequence
  Description of Artificial Sequence: Synthetic peptide
DRYSSSNHYNGMDV

SEQ ID NO: 13 - protein, 5 aa, Artificial Sequence
  Description of Artificial Sequence: Synthetic peptide
SYAMT

SEQ ID NO: 14 - protein, 17 aa, Artificial Sequence
  Description of Artificial Sequence: Synthetic peptide
VISGSGGSTYYADSVKG

SEQ ID NO: 15 - protein, 16 aa, Artificial Sequence
  Description of Artificial Sequence: Synthetic peptide
DGRQVEDYYYYYGMDV

SEQ ID NO: 16 - protein, 14 aa, Artificial Sequence
  Description of Artificial Sequence: Synthetic peptide
DRYSPTGHYMGMDV

SEQ ID NO: 17 - protein, 16 aa, Artificial Sequence
  Description of Artificial Sequence: Synthetic peptide
VIDTAGDTYYPGSVKG

SEQ ID NO: 18 - protein, 14 aa, Artificial Sequence
  Description of Artificial Sequence: Synthetic peptide
DRYSGNFHYNGMDV

SEQ ID NO: 19 - protein, 106 aa, Artificial Sequence
  Description of Artificial Sequence: Synthetic polypeptide
DIQMTQSPSTLSASVGDRVTITCRASQSISSWLAWYQQKPGKAPKLLIYKASSLESGVPSRFSGSGSGTEFTLTISSLQPDDFATYYCQQYNSYWTFGQGTKVEIK

SEQ ID NO: 20 - protein, 122 aa, Artificial Sequence
  Description of Artificial Sequence: Synthetic polypeptide
EVQLVESGGGLVQPGGSLRLSCAASGFTFSSYDMHWVRQATGKGLEWVSGIGTAGDTYYPGSVKGRFTISRENAKNSLYLQLNSLRAGDTAVYFCARDNYSSTGGYYGMDVWGQGTTVTVSS

SEQ ID NO: 21 - protein, 106 aa, Artificial Sequence; identical to SEQ ID NO: 19
  Description of Artificial Sequence: Synthetic polypeptide

SEQ ID NO: 22 - protein, 122 aa, Artificial Sequence
  Description of Artificial Sequence: Synthetic polypeptide
EVQLVESGGGLVQPGGSLRLSCAASGFTFSRYDMHWVRQATGKGLEWVSVIGTDGDTYYPGSVKGRFIISRENAKNSLYLEMNSLRAGDTAVYYCARDRYSSSNHYNGMDVWGQGTTVTVSS

SEQ ID NO: 23 - protein, 106 aa, Artificial Sequence
  Description of Artificial Sequence: Synthetic polypeptide
DIQMTQSPSTLSASVGDRVTITCRASQSISSWLAWYQQKPGKAPKVLIYKASSLESGVPSRFSGSGSGTEFTLTISSLQPDDFATYYCQQYNSYWTFGQGTKVEIK

SEQ ID NO: 24 - protein, 122 aa, Artificial Sequence; identical to SEQ ID NO: 22
  Description of Artificial Sequence: Synthetic polypeptide

SEQ ID NO: 25 - protein, 107 aa, Artificial Sequence
  Description of Artificial Sequence: Synthetic polypeptide
AIQMTQSPSSLSASVGDRVTITCRASQGIRNDLGWYQQKPGKAPKLLIYDASSLQSGVPSRFSGSGSGTDFTLTISSLQPEDFATYYCLQDYNYPWTFGQGTKVEIK

SEQ ID NO: 26 - protein, 125 aa, Artificial Sequence
  Description of Artificial Sequence: Synthetic polypeptide
EVQLLESGGGLVQPGGSLRLSCAASGFTFSSYAMTWVRQAPGKGLEWVSVISGSGGSTYYADSVKGRFTVSRDNSKNTLYLQMNSLRAEDTAVYYCAKDGRQVEDYYYYYGMDVWGQGTTVTVSS

SEQ ID NO: 27 - protein, 106 aa, Artificial Sequence; identical to SEQ ID NO: 19
  Description of Artificial Sequence: Synthetic polypeptide

SEQ ID NO: 28 - protein, 122 aa, Artificial Sequence
  Description of Artificial Sequence: Synthetic polypeptide
EVQLVESGGGLVQPGGSLRLSCTASGFTFSSYDMHWVRQATGKGLEWVSVIDTAGDTYYPGSVKGRFTISRENAKNSLYLQMNSLRAGDTAVYYCVRDRYSGNFHYNGMDVWGQGTTVTVSS

SEQ ID NO: 29 - protein, 122 aa, Artificial Sequence
  Description of Artificial Sequence: Synthetic polypeptide
EVQLVESGGGLVQPGGSLRLSCAASGFTFSSYDMHWVRQATGKGLEWVSGIGTAGDTYYPGSVKGRFTISRENAKNSLYLQMNSLRAGDTAVYYCARDRYSPTGHYMGMDVWGQGTTVTVSS

SEQ ID NO: 30 - protein, 106 aa, Artificial Sequence
  Description of Artificial Sequence: Synthetic polypeptide
DIQMTQSPSTLSASVGDRVTITCRASQSISSWLAWYQQKPGKAPKLLIYKASSLESGVPSRFSGSGSGTEFTLTISSLQPDDFATYYCQQYDTYWTFGQGTKVEIK

SEQ ID NO: 31 - protein, 122 aa, Artificial Sequence
  Description of Artificial Sequence: Synthetic polypeptide
EVQLVESGGGLVQPGGSLRLSCAASGFTFSSYDMHWVRQATGKGLEWVSGIGTAGDTYYPGSVKGRFTISRENAKNSLYLQMNSLRAGDTAVYYCARDRYSRTGHYMGMDVWGQGTTVTVSS

SEQ ID NO: 32 - protein, 106 aa, Artificial Sequence; identical to SEQ ID NO: 30
  Description of Artificial Sequence: Synthetic polypeptide

SEQ ID NO: 33 - protein, 122 aa, Artificial Sequence
  Description of Artificial Sequence: Synthetic polypeptide
EVQLVESGGGLVQPGGSLRLSCAASGFTFSSYDMHWVRQATGKGLEWVSGIGTAGDTYYPGSVKGRFTISRENAKNSLYLQMNSLRAGDTAVYYCARDRYSRTGHYMGMSLWGQGTTVTVSS

SEQ ID NO: 34 - protein, 106 aa, Artificial Sequence; identical to SEQ ID NO: 30
  Description of Artificial Sequence: Synthetic polypeptide

SEQ ID NO: 35 - protein, 122 aa, Artificial Sequence
  Description of Artificial Sequence: Synthetic polypeptide
EVQLVESGGGLVQPGGSLRLSCAASGFTFSSYDMHWVRQATGKGLEWVSGIGTAGDTYYPGSVKGRFTISRENAKNSLYLQMNSLRAGDTAVYYCARDNYSRTGHYMGMDVWGQGTTVTVSS

SEQ ID NO: 36 - protein, 106 aa, Artificial Sequence
  Description of Artificial Sequence: Synthetic polypeptide
DIQMTQSPSTLSASVGDRVTITCRASQSISSWLAWYQQKPGKAPKLLIYKASSLESGVPSRFSGSGSGTEFTLTISSLQPDDFATYYCKQYADYWTFGQGTKVEIK

SEQ ID NO: 37 - protein, 122 aa, Artificial Sequence; identical to SEQ ID NO: 35
  Description of Artificial Sequence: Synthetic polypeptide

SEQ ID NO: 38 - protein, 106 aa, Artificial Sequence; identical to SEQ ID NO: 30
  Description of Artificial Sequence: Synthetic polypeptide

SEQ ID NO: 39 - protein, 122 aa, Artificial Sequence
  Description of Artificial Sequence: Synthetic polypeptide
EVQLVESGGGLVQPGGSLRLSCAASGFTFSSYDMHWVRQATGKGLEWVSGIGTAGDTYYPGSVKGRFTISRENAKNSLYLQMNSLRAGDTAVYYCARDRYSPTGHYMGMSLWGQGTTVTVSS

SEQ ID NO: 40 - protein, 106 aa, Artificial Sequence; identical to SEQ ID NO: 30
  Description of Artificial Sequence: Synthetic polypeptide

SEQ ID NO: 41 - protein, 122 aa, Artificial Sequence; identical to SEQ ID NO: 31
  Description of Artificial Sequence: Synthetic polypeptide

SEQ ID NO: 42 - protein, 106 aa, Artificial Sequence; identical to SEQ ID NO: 36
  Description of Artificial Sequence: Synthetic polypeptide

SEQ ID NO: 43 - protein, 122 aa, Artificial Sequence
  Description of Artificial Sequence: Synthetic polypeptide
EVQLVESGGGLVQPGGSLRLSCAASGFTFSSYDMHWVRQATGKGLEWVSGIGTAGDTYYPGSVKGRFTISRENAKNSLYLQMNSLRAGDTAVYYCARDNYSSTGGYYGMDVWGQGTTVTVSS

SEQ ID NO: 44 - protein, 106 aa, Artificial Sequence; identical to SEQ ID NO: 19
  Description of Artificial Sequence: Synthetic polypeptide

SEQ ID NO: 45 - protein, 122 aa, Artificial Sequence
  Description of Artificial Sequence: Synthetic polypeptide
EVQLVESGGGLVQPGGSLRLSCAASGFTFSSHDMHWVRQATGKGLEWVSGIGTAGDTYYPDSVKGRFTISRENAKNSLYLQMNSLRAGDTAVYYCARDRYSPTGHYYGMDVWGQGTTVTVSS

SEQ ID NO: 46 - protein, 106 aa, Artificial Sequence; identical to SEQ ID NO: 36
  Description of Artificial Sequence: Synthetic polypeptide

SEQ ID NO: 47 - protein, 122 aa, Artificial Sequence
  Description of Artificial Sequence: Synthetic polypeptide
EVQLVESGGGLVQPGGSLRLSCAASGFTFSSYDMHWVRQATGKGLEWVSGIGTAGDTYYPGSVKGRFTISRENAKNSLYLQMNSLRAGDTAVYYCARDNYSPTGGYYGMDVWGQGTTVTVSS

SEQ ID NO: 48 - protein, 106 aa, Artificial Sequence
  Description of Artificial Sequence: Synthetic polypeptide
DIQMTQSPSTLSASVGDRVTITCRASQSISSWLAWYQQKPGKAPKLLIYKASSLKSGVPSRFSGSGSGTEFTLTISSLQPDDFATYYCQQYESYWTFGQGTKVEIK

SEQ ID NO: 49 - protein, 122 aa, Artificial Sequence
  Description of Artificial Sequence: Synthetic polypeptide
EVQLVESGGGLVQPGGSLRLSCAASGFTFSSHDMHWVRQATGKGLEWVSGIGTRGDTYYPDSVKGRFTISRENAKNSLYLQMNSLRAGDTAVYYCARDRYSPTGHYYGMDVWGQGTTVTVSS

SEQ ID NO: 50 - protein, 122 aa, Artificial Sequence
  Description of Artificial Sequence: Synthetic polypeptide
EVQLVESGGGLVQPGGSLRLSCAASGFTFSSHDMHWVRQATGKGLEWVSGIGTRGDTYYPDSVKGRFTISRENAKNSLYLQMNSLRAGDTAVYYCARDKYSPTGHYYGMDVWGQGTTVTVSS

SEQ ID NO: 51 - protein, 106 aa, Artificial Sequence
  Description of Artificial Sequence: Synthetic polypeptide
DIQMTQSPSTLSASVGDRVTITCRASQSISSWLAWYQQKPGKAPKLLIYKASSLVKGVPSRFSGSGSGTEFTLTISSLQPDDFATYYCQQYESYWTFGQGTKVEIK

SEQ ID NO: 52 - protein, 8 aa, Artificial Sequence
  Description of Artificial Sequence: Synthetic peptide
QQYDTYWT

SEQ ID NO: 53 - protein, 14 aa, Artificial Sequence
  Description of Artificial Sequence: Synthetic peptide
DRYSRTGHYMGMDV

SEQ ID NO: 54 - protein, 14 aa, Artificial Sequence
  Description of Artificial Sequence: Synthetic peptide
DRYSRTGHYMGMSL

SEQ ID NO: 55 - protein, 14 aa, Artificial Sequence
  Description of Artificial Sequence: Synthetic peptide
DNYSRTGHYMGMDV

SEQ ID NO: 56 - protein, 8 aa, Artificial Sequence
  Description of Artificial Sequence: Synthetic peptide
KQYADYWT

SEQ ID NO: 57 - protein, 5 aa, Artificial Sequence
  Description of Artificial Sequence: Synthetic peptide
SHDMH

SEQ ID NO: 58 - protein, 16 aa, Artificial Sequence
  Description of Artificial Sequence: Synthetic peptide
GIGTAGDTYYPDSVKG

SEQ ID NO: 59 - protein, 14 aa, Artificial Sequence
  Description of Artificial Sequence: Synthetic peptide
DRYSPTGHYYGMDV

SEQ ID NO: 60 - protein, 14 aa, Artificial Sequence
  Description of Artificial Sequence: Synthetic peptide
DNYSPTGGYYGMDV

SEQ ID NO: 61 - protein, 7 aa, Artificial Sequence
  Description of Artificial Sequence: Synthetic peptide
KASSLKS

SEQ ID NO: 62 - protein, 8 aa, Artificial Sequence
  Description of Artificial Sequence: Synthetic peptide
QQYESYWT

SEQ ID NO: 63 - protein, 16 aa, Artificial Sequence
  Description of Artificial Sequence: Synthetic peptide
GIGTRGDTYYPDSVKG

SEQ ID NO: 64 - protein, 14 aa, Artificial Sequence
  Description of Artificial Sequence: Synthetic peptide
DKYSPTGHYYGMDV

SEQ ID NO: 65 - protein, 7 aa, Artificial Sequence
  Description of Artificial Sequence: Synthetic peptide
KASSLVK

SEQ ID NO: 66 - protein, 14 aa, Artificial Sequence
  Description of Artificial Sequence: Synthetic peptide
DRYSPTGHYMGMSL

SEQ ID NO: 67 - protein, 122 aa, Artificial Sequence; identical to SEQ ID NO: 45
  Description of Artificial Sequence: Synthetic polypeptide

SEQ ID NO: 68 - protein, 452 aa, Artificial Sequence
  Description of Artificial Sequence: Synthetic polypeptide
EVQLVESGGGLVQPGGSLRLSCAASGFTFSSHDMHWVRQATGKGLEWVSGIGTAGDTYYPDSVKGRFTISRENAKNSLYLQMNSLRAGDTAVYYCARDRYSPTGHYYGMDVWGQGTTVTVSSASTKGPSVFPLAPSSKSTSGGTAALGCLVKDYFPEPVTVSWNSGALTSGVHTFPAVLQSSGLYSLSSVVTVPSSSLGTQTYICNVNHKPSNTKVDKRVEPKSCDKTHTCPPCPAPELLGGPSVFLFPPKPKDTLYITREPEVTCVVVDVSHEDPEVKFNWYVDGVEVHNAKTKPREEQYNSTYRVVSVLTVLHQDWLNGKEYKCKVSNKALPAPIEKTISKAKGQPREPQVYTLPPSREEMTKNQVSLTCLVKGFYPSDIAVEWESNGQPENNYKTTPPVLDSDGSFFLYSKLTVDKSRWQQGNVFSCSVMHEALHNHYTQKSLSLSPGK

SEQ ID NO: 69 - protein, 212 aa, Artificial Sequence
  Description of Artificial Sequence: Synthetic polypeptide
DIQMTQSPSTLSASVGDRVTITCRASQSISSWLAWYQQKPGKAPKLLIYKASSLESGVPSRFSGSGSGTEFTLTISSLQPDDFATYYCKQYADYWTFGQGTKVEIKRTVAAPSVFIFPPSDEQLKSGTASVVCLLNNFYPREAKVQWKVDNALQSGNSQESVTEQDSKDSTYSLSSTLTLSKADYEKHKVYACEVTHQGLSSPVTKSFNRGE

SEQ ID NO: 70 - protein, 293 aa, Staphylococcus aureus
ADSDINIKTGTTDIGSNTTVKTGDLVTYDKENGMHKKVFYSFIDDKNHNKKLLVIRTKGTIAGQYRVYSEEGANKSGLAWPSAFKVQLQLPDNEVAQISDYYPRNSIDTKEYMSTLTYGFNGNVTGDDTGKIGGLIGANVSIGHTLKYVQPDFKTILESPTDKKVGWKVIFNNMVNQNWGPYDRDSWNPVYGNQLFMKTRNGSMKAADNFLDPNKASSLLSSGFSPDFATVITMDRKASKQQTNIDVIYERVRDDYQLHWTSTNWKGTNTKDKWTDRSSERYKIDWEKEEMTN

SEQ ID NO: 71 - protein, 119 aa, Artificial
  WapR-004 VH
EVQLLESGPGLVKPSETLSLTCNVAGGSISPYYWTWIRQPPGKGLELIGYIHSSGYTDYNPSLKSRVTISGDTSKKQFSLHVSSVTAADTAVYFCARGDWDLLHALDIWGQGTLVTVSS

SEQ ID NO: 72 - protein, 107 aa, Artificial
  WapR-004 & WarR-004RAD VL
EIVLTQSPSSLSTSVGDRVTITCRASQSIRSHLNWYQQKPGKAPKLLIYGASNLQSGVPSRFSGSGSGTDFTLTISSLQPEDFATYYCQQSYSFPLTFGGGTKLEIK

SEQ ID NO: 73 - protein, 5 aa, Artificial
  WapR-004 & WapR-004RAD VHCDR1
PYYWT

SEQ ID NO: 74 - protein, 16 aa, Artificial
  WapR-004 & WapR-004RAD VHCDR2
YIHSSGYTDYNPSLKS

SEQ ID NO: 75 - protein, 11 aa, Artificial
  WapR-004 VHCDR3
GDWDLLHALDI

SEQ ID NO: 76 - protein, 11 aa, Artificial
  WapR-004 & WapR-004RAD VLCDR1
RASQSIRSHLN

SEQ ID NO: 77 - protein, 7 aa, Artificial
  WapR-004 & WapR-004RAD VLCDR2
GASNLQS

SEQ ID NO: 78 - protein, 6 aa, Artificial
  WapR-004 & WapR-004RAD VLCDR3
YSFPLT

SEQ ID NO: 79 - protein, 119 aa, Artificial
  WapR-004RAD VH
EVQLLESGPGLVKPSETLSLTCNVAGGSISPYYWTWIRQPPGKGLELIGYIHSSGYTDYNPSLKSRVTISGDTSKKQFSLHVSSVTAADTAVYFCARADWDLLHALDIWGQGTLVTVSS

SEQ ID NO: 80 - protein, 11 aa, Artificial
  WapR-004RAD VHCDR3
ADWDLLHALDI

SEQ ID NO: 81 - protein, 124 aa, Artificial
  V2L2 VH
EMQLLESGGGLVQPGGSLRLSCAASGFTFSSYAMNWVRQAPGEGLEWVSAITISGITAYYTDSVKGRFTISRDNSKNTLYLQMNSLRAGDTAVYYCAKEEFLPGTHYYYGMDVWGQGTTVTVSS

SEQ ID NO: 82 - protein, 107 aa, Artificial
  V2L2 VL
AIQMTQSPSSLSASVGDRVTITCRASQGIRNDLGWYQQKPGKAPKLVIYSASTLQSGVPSRFSGSGSGTDFTLSISSLQPDDFATYYCLQDYNYPWTFGQGTKVEIK

SEQ ID NO: 83 - protein, 5 aa, Artificial
  V2L2  VHCDR1
SYAMN

SEQ ID NO: 84 - protein, 17 aa, Artificial
  V2L2  VHCDR2
AITISGITAYYTDSVKG

SEQ ID NO: 85 - protein, 15 aa, Artificial
  V2L2  VHCDR3
EEFLPGTHYYYGMDV

SEQ ID NO: 86 - protein, 11 aa, Artificial
  V2L2  VLCDR1
RASQGIRNDLG

SEQ ID NO: 87 - protein, 7 aa, Artificial
  V2LC  VLCDR2
SASTLQS

SEQ ID NO: 88 - protein, 9 aa, Artificial
  V2L2  VLCDR3
LQDYNYPWT

SEQ ID NO: 89 - protein, 256 aa, Artificial
  W4-RAD scFv sequence in BS3 vector
GGGGSGGGGSEVQLLESGPGLVKPSETLSLTCNVAGGSISPYYWTWIRQPPGKCLELIGYIHSSGYTDYNPSLKSRVTISGDTSKKQFSLHVSSVTAADTAVYFCARADWDLLHALDIWGQGTLVTVSSGGGGSGGGGSGGGGSGGGGSEIVLTQSPSSLSTSVGDRVTITCRASQSIRSHLNWYQQKPGKAPKLLIYGASNLQSGVPSRFSGSGSGTDFTLTISSLQPEDFATYYCQQSYSFPLTFGCGTKLEIK

SEQ ID NO: 90 - protein, 380 aa, Artificial
  W4-RAD scFv-V2L2 VH sequences in Bs2 vector
EVQLLESGPGLVKPSETLSLTCNVAGGSISPYYWTWIRQPPGKCLELIGYIHSSGYTDYNPSLKSRVTISGDTSKKQFSLHVSSVTAADTAVYFCARADWDLLHALDIWGQGTLVTVSSGGGGSGGGGSGGGGSGGGGSEIVLTQSPSSLSTSVGDRVTITCRASQSIRSHLNWYQQKPGKAPKLLIYGASNLQSGVPSRFSGSGSGTDFTLTISSLQPEDFATYYCQQSYSFPLTFGCGTKLEIKGGGGSGGGGSEMQLLESGGGLVQPGGSLRLSCAASGFTFSSYAMNWVRQAPGEGLEWVSAITISGITAYYTDSVKGRFTISRDNSKNTLYLQMNSLRAGDTAVYYCAKEEFLPGTHYYYGMDVWGQGTTVTVSS

SEQ ID NO: 91 - protein, 292 aa, Artificial
  W4-RAD scFv in Bs4 vector
KVDKRVEPKSCGGGGSGGGGSEVQLLESGPGLVKPSETLSLTCNVAGGSISPYYWTWIRQPPGKCLELIGYIHSSGYTDYNPSLKSRVTISGDTSKKQFSLHVSSVTAADTAVYFCARADWDLLHALDIWGQGTLVTVSSGGGGSGGGGSGGGGSGGGGSEIVLTQSPSSLSTSVGDRVTITCRASQSIRSHLNWYQQKPGKAPKLLIYGASNLQSGVPSRFSGSGSGTDFTLTISSLQPEDFATYYCQQSYSFPLTFGCGTKLEIKGGGGSGGGGSDKTHTCPPCPAPELL

SEQ ID NO: 92 - protein, 214 aa, Artificial
  Bs4-V2L2-C2 light
AIQMTQSPSSLSASVGDRVTITCRASQGIRNDLGWYQQKPGKAPKLVIYSASTLQSGVPSRFSGSGSGTDFTLSISSLQPDDFATYYCLQDYNYPWTFGQGTKVEIKRTVAAPSVFIFPPSDEQLKSGTASVVCLLNNFYPREAKVQWKVDNALQSGNSQESVTEQDSKDSTYSLSSTLTLSKADYEKHKVYACEVTHQGLSSPVTKSFNRGEC

SEQ ID NO: 93 - protein, 720 aa, Artificial
  Bs4-V2L2-C2 heavy
EMQLLESGGGLVQPGGSLRLSCAASGFTFSSYAMNWVRQAPGEGLEWVSAITISGITAYYTDSVKGRFTISRDNSKNTLYLQMNSLRAGDTAVYYCAKEEFLPGTHYYYGMDVWGQGTTVTVSSASTKGPSVFPLAPSSKSTSGGTAALGCLVKDYFPEPVTVSWNSGALTSGVHTFPAVLQSSGLYSLSSVVTVPSSSLGTQTYICNVNHKPSNTKVDKRVEPKSCGGGGSGGGGSEVQLLESGPGLVKPSETLSLTCNVAGGSISPYYWTWIRQPPGKCLELIGYIHSSGYTDYNPSLKSRVTISGDTSKKQFSLHVSSVTAADTAVYFCARADWDLLHALDIWGQGTLVTVSSGGGGSGGGGSGGGGSGGGGSEIVLTQSPSSLSTSVGDRVTITCRASQSIRSHLNWYQQKPGKAPKLLIYGASNLQSGVPSRFSGSGSGTDFTLTISSLQPEDFATYYCQQSYSFPLTFGCGTKLEIKGGGGSGGGGSDKTHTCPPCPAPELLGGPSVFLFPPKPKDTLMISRTPEVTCVVVDVSHEDPEVKFNWYVDGVEVHNAKTKPREEQYNSTYRVVSVLTVLHQDWLNGKEYKCKVSNKALPAPIEKTISKAKGQPREPQVYTLPPSREEMTKNQVSLTCLVKGFYPSDIAVEWESNGQPENNYKTTPPVLDSDGSFFLYSKLTVDKSRWQQGNVFSCSVMHEALHNHYTQKSLSLSPGK

SEQ ID NO: 94 - protein, 11 aa, Artificial
  Psl0096-Germline VHCDR3
ADWDRLRALDI

SEQ ID NO: 95 - protein, 9 aa, Artificial
  Psl0096-Germline VLCDR3
QQSTGAWNW

SEQ ID NO: 96 - protein, 119 aa, Artificial
  Psl0096-Germline VH
  misc_feature (44)..(44): Xaa is Gly or Cys
QVQLQESGPGLVKPSETLSLTCTVSGGSISPYYWTWIRQPPGKXLELIGYIHSSGYTDYNPSLKSRVTISGDTSKKQFSLKLSSVTAADTAVYYCARADWDRLRALDIWGQGTMVTVSS

SEQ ID NO: 97 - protein, 107 aa, Artificial
  Psl0096-Germline VL
  misc_feature (100)..(100): Xaa can be Gly or Cys
DIQLTQSPSSLSASVGDRVTITCRASQSIRSHLNWYQQKPGKAPKLLIYGASNLQSGVPSRFSGSGSGTDFTLTISSLQPEDFATYYCQQSTGAWNWFGXGTKVEIK

SEQ ID NO: 98 - protein, 124 aa, Artificial; identical to SEQ ID NO: 81
  V2L2-MD VH

SEQ ID NO: 99 - protein, 107 aa, Artificial; identical to SEQ ID NO: 82
  V2L2-MD VL

SEQ ID NO: 100 - protein, 214 aa, Artificial
  Bs4-GLO LC
AIQMTQSPSSLSASVGDRVTITCRASQGIRNDLGWYQQKPGKAPKLLIYSASTLQSGVPSRFSGSGSGTDFTLTISSLQPEDFATYYCLQDYNYPWTFGQGTKVEIKRTVAAPSVFIFPPSDEQLKSGTASVVCLLNNFYPREAKVQWKVDNALQSGNSQESVTEQDSKDSTYSLSSTLTLSKADYEKHKVYACEVTHQGLSSPVTKSFNRGEC

SEQ ID NO: 101 - protein, 720 aa, Artificial [sequence omitted]